European Patent Application EP 4 752 161 A1, published June 3, 2026. Title: FUSION PROTEIN FOR THE TREATMENT OF DISEASES ASSOCIATED WITH CD20. Applicant: 上海药明巨诺生物医药研发有限公司. The sequence listing filed with the application follows.

SEQUENCE LISTING (43 sequences)

SEQ ID NO: 1 - protein, 247 aa, synthetic construct
EVQLVESGGGLVQPGRSLRLSCAASGFTFNDYAMHWVRQAPGKGLEWVSTISWNSGSIGYADSVKGRFTISRDNAKKSLYLQMNSLRAEDTALYYCAKDIQYGNYYYGMDVWGQGTTVTVSSGGGGSGGGGSGGGGSEIVLTQSPATLSLSPGERATLSCRASQSVSSYLAWYQQKPGQAPRLLIYDASNRATGIPARFSGSGSGTDFTLTISSLEPEDFAVYYCQQRSNWPITFGQGTRLEIKRTV

SEQ ID NO: 2 - protein, 249 aa, synthetic construct
QVQLVQSGAEVKKPGSSVKVSCKASGYAFSYSWINWVRQAPGQGLEWMGRIFPGDGDTDYNGKFKGRVTITADKSTSTAYMELSSLRSEDTAVYYCARNVFDGYWLVYWGQGTLVTVSSGGGGSGGGGSGGGGSDIVMTQTPLSLPVTPGEPASISCRSSKSLLHSNGITYLYWYLQKPGQSPQLLIYQMSNLVSGVPDRFSGSGSGTDFTLKISRVEAEDVGVYYCAQNLELPYTFGGGTKVEIKRTV

SEQ ID NO: 3 - protein, 242 aa, synthetic construct
QVQLQQPGAELVKPGASVKMSCKASGYTFTSYNMHWVKQTPGRGLEWIGAIYPGNGDTSYNQKFKGKATLTADKSSSTAYMQLSSLTSEDSAVYYCARSTYYGGDWYFNVWGAGTTVTVSGGGGSGGGGSGGGGSQIVLSQSPAILSASPGEKVTMTCRASSSVSYIHWFQQKPGSSPKPWIYATSNLASGVPVRFSGSGSGTSYSLTISRVEAEDAATYYCQQWTSNPPTFGGGTKLEIKR

SEQ ID NO: 4 - protein, 122 aa, synthetic construct
EVQLVESGGGLVQPGRSLRLSCAASGFTFNDYAMHWVRQAPGKGLEWVSTISWNSGSIGYADSVKGRFTISRDNAKKSLYLQMNSLRAEDTALYYCAKDIQYGNYYYGMDVWGQGTTVTVSS

SEQ ID NO: 5 - protein, 110 aa, synthetic construct
EIVLTQSPATLSLSPGERATLSCRASQSVSSYLAWYQQKPGQAPRLLIYDASNRATGIPARFSGSGSGTDFTLTISSLEPEDFAVYYCQQRSNWPITFGQGTRLEIKRTV

SEQ ID NO: 6 - protein, 5 aa, synthetic construct
DYAMH

SEQ ID NO: 7 - protein, 17 aa, synthetic construct
TISWNSGSIGYADSVKG

SEQ ID NO: 8 - protein, 13 aa, synthetic construct
DIQYGNYYYGMDV

SEQ ID NO: 9 - protein, 11 aa, synthetic construct
RASQSVSSYLA

SEQ ID NO: 10 - protein, 7 aa, synthetic construct
DASNRAT

SEQ ID NO: 11 - protein, 9 aa, synthetic construct
QQRSNWPIT

SEQ ID NO: 12 - protein, 119 aa, synthetic construct
QVQLVQSGAEVKKPGSSVKVSCKASGYAFSYSWINWVRQAPGQGLEWMGRIFPGDGDTDYNGKFKGRVTITADKSTSTAYMELSSLRSEDTAVYYCARNVFDGYWLVYWGQGTLVTVSS

SEQ ID NO: 13 - protein, 115 aa, synthetic construct
DIVMTQTPLSLPVTPGEPASISCRSSKSLLHSNGITYLYWYLQKPGQSPQLLIYQMSNLVSGVPDRFSGSGSGTDFTLKISRVEAEDVGVYYCAQNLELPYTFGGGTKVEIKRTV

SEQ ID NO: 14 - protein, 5 aa, synthetic construct
YSWIN

SEQ ID NO: 15 - protein, 17 aa, synthetic construct
RIFPGDGDTDYNGKFKG

SEQ ID NO: 16 - protein, 10 aa, synthetic construct
NVFDGYWLVY

SEQ ID NO: 17 - protein, 16 aa, synthetic construct
RSSKSLLHSNGITYLY

SEQ ID NO: 18 - protein, 7 aa, synthetic construct
QMSNLVS

SEQ ID NO: 19 - protein, 9 aa, synthetic construct
AQNLELPYT

SEQ ID NO: 20 - protein, 120 aa, synthetic construct
QVQLQQPGAELVKPGASVKMSCKASGYTFTSYNMHWVKQTPGRGLEWIGAIYPGNGDTSYNQKFKGKATLTADKSSSTAYMQLSSLTSEDSAVYYCARSTYYGGDWYFNVWGAGTTVTVS

SEQ ID NO: 21 - protein, 107 aa, synthetic construct
QIVLSQSPAILSASPGEKVTMTCRASSSVSYIHWFQQKPGSSPKPWIYATSNLASGVPVRFSGSGSGTSYSLTISRVEAEDAATYYCQQWTSNPPTFGGGTKLEIKR

SEQ ID NO: 22 - protein, 5 aa, synthetic construct
SYNMH

SEQ ID NO: 23 - protein, 17 aa, synthetic construct
AIYPGNGDTSYNQKFKG

SEQ ID NO: 24 - protein, 12 aa, synthetic construct
STYYGGDWYFNV

SEQ ID NO: 25 - protein, 10 aa, synthetic construct
RASSSVSYIH

SEQ ID NO: 26 - protein, 7 aa, synthetic construct
ATSNLAS

SEQ ID NO: 27 - protein, 9 aa, synthetic construct
QQWTSNPPT

SEQ ID NO: 28 - protein, 15 aa, synthetic construct
GGGGSGGGGSGGGGS

SEQ ID NO: 29 - protein, 38 aa, synthetic construct
PPTPAPTIASQPLSLRPEACRPAAGGAVHTRGLDFACD

SEQ ID NO: 30 - protein, 40 aa, synthetic construct
KIEVMYPPPYLDNEKSNGTIIHVKGKHLCPSPLFPGPSKP

SEQ ID NO: 31 - protein, 12 aa, synthetic construct
ESKYGPPCPPCP

SEQ ID NO: 32 - protein, 24 aa, synthetic construct
IYIWAPLAGTCGVLLLSLVITLYC

SEQ ID NO: 33 - protein, 28 aa, synthetic construct
MFWVLVVVGGVLACYSLLVTVAFIIFWV

SEQ ID NO: 34 - protein, 42 aa, synthetic construct
KRGRKKLLYIFKQPFMRPVQTTQEEDGCSCRFPEEEEGGCEL

SEQ ID NO: 35 - protein, 112 aa, synthetic construct
RVKFSRSADAPAYQQGQNQLYNELNLGRREEYDVLDKRRGRDPEMGGKPRRKNPQEGLYNELQKDKMAEAYSEIGMKGERRRGKGHDGLYQGLSTATKDTYDALHMQALPPR

SEQ ID NO: 36 - protein, 469 aa, synthetic construct
EVQLVESGGGLVQPGRSLRLSCAASGFTFNDYAMHWVRQAPGKGLEWVSTISWNSGSIGYADSVKGRFTISRDNAKKSLYLQMNSLRAEDTALYYCAKDIQYGNYYYGMDVWGQGTTVTVSSGGGGSGGGGSGGGGSEIVLTQSPATLSLSPGERATLSCRASQSVSSYLAWYQQKPGQAPRLLIYDASNRATGIPARFSGSGSGTDFTLTISSLEPEDFAVYYCQQRSNWPITFGQGTRLEIKRTVKIEVMYPPPYLDNEKSNGTIIHVKGKHLCPSPLFPGPSKPMFWVLVVVGGVLACYSLLVTVAFIIFWVKRGRKKLLYIFKQPFMRPVQTTQEEDGCSCRFPEEEEGGCELRVKFSRSADAPAYQQGQNQLYNELNLGRREEYDVLDKRRGRDPEMGGKPRRKNPQEGLYNELQKDKMAEAYSEIGMKGERRRGKGHDGLYQGLSTATKDTYDALHMQALPPR

SEQ ID NO: 37 - protein, 443 aa, synthetic construct
QVQLVQSGAEVKKPGSSVKVSCKASGYAFSYSWINWVRQAPGQGLEWMGRIFPGDGDTDYNGKFKGRVTITADKSTSTAYMELSSLRSEDTAVYYCARNVFDGYWLVYWGQGTLVTVSSGGGGSGGGGSGGGGSDIVMTQTPLSLPVTPGEPASISCRSSKSLLHSNGITYLYWYLQKPGQSPQLLIYQMSNLVSGVPDRFSGSGSGTDFTLKISRVEAEDVGVYYCAQNLELPYTFGGGTKVEIKRTVESKYGPPCPPCPMFWVLVVVGGVLACYSLLVTVAFIIFWVKRGRKKLLYIFKQPFMRPVQTTQEEDGCSCRFPEEEEGGCELRVKFSRSADAPAYQQGQNQLYNELNLGRREEYDVLDKRRGRDPEMGGKPRRKNPQEGLYNELQKDKMAEAYSEIGMKGERRRGKGHDGLYQGLSTATKDTYDALHMQALPPR

SEQ ID NO: 38 - protein, 441 aa, synthetic construct
EVQLVESGGGLVQPGRSLRLSCAASGFTFNDYAMHWVRQAPGKGLEWVSTISWNSGSIGYADSVKGRFTISRDNAKKSLYLQMNSLRAEDTALYYCAKDIQYGNYYYGMDVWGQGTTVTVSSGGGGSGGGGSGGGGSEIVLTQSPATLSLSPGERATLSCRASQSVSSYLAWYQQKPGQAPRLLIYDASNRATGIPARFSGSGSGTDFTLTISSLEPEDFAVYYCQQRSNWPITFGQGTRLEIKRTVESKYGPPCPPCPMFWVLVVVGGVLACYSLLVTVAFIIFWVKRGRKKLLYIFKQPFMRPVQTTQEEDGCSCRFPEEEEGGCELRVKFSRSADAPAYQQGQNQLYNELNLGRREEYDVLDKRRGRDPEMGGKPRRKNPQEGLYNELQKDKMAEAYSEIGMKGERRRGKGHDGLYQGLSTATKDTYDALHMQALPPR

SEQ ID NO: 39 - protein, 20 aa, synthetic construct
METDTLLLWVLLLWVPGSTG

SEQ ID NO: 40 - protein, 357 aa, synthetic construct
MLLLVTSLLLCELPHPAFLLIPRKVCNGIGIGEFKDSLSINATNIKHFKNCTSISGDLHILPVAFRGDSFTHTPPLDPQELDILKTVKEITGFLLIQAWPENRTDLHAFENLEIIRGRTKQHGQFSLAVVSLNITSLGLRSLKEISDGDVIISGNKNLCYANTINWKKLFGTSGQKTKIISNRGENSCKATGQVCHALCSPEGCWGPEPRDCVSCRNVSRGRECVDKCNLLEGEPREFVENSECIQCHPECLPQAMNITCTGRGPDNCIQCAHYIDGPHCVKTCPAGVMGENNTLVWKYADAGHVCHLCHPNCTYGCTGPGLEGCPTNGPKIPSIATGMVGALLLLLVVALGIGLFM

SEQ ID NO: 41 - protein, 5 aa, synthetic construct
  REPEAT 1..5: note = Repeated for 1, 2, 3, 4, 5, 6, 7 or 8, in particular 3 times
GGGGS

SEQ ID NO: 42 - protein, 5 aa, synthetic construct
  REPEAT 1..5: note = Repeated for 1, 2, 3, 4, 5, 6, 7 or 8, in particular 3 times
SGGGG

SEQ ID NO: 43 - protein, 9 aa, synthetic construct
  REPEAT 5..9: note = Repeated for 1, 2, 3, 4, 5, 6, 7 or 8, in particular 3 times
GGGGSGGGG